European Patent Application EP 4 793 350 A1, published August 19, 2026. Title: FUSION PROTEINS AND THE USE THEREOF FOR THE TREATMENT OF CORONAVIRUS INFECTIONS. Applicant: FUNDACIÓ PRIVADA INSTITUT DE RECERCA SOBRE IMMUNOPATOLOGIES-CAIXA IRSICAIXA. The sequence listing filed with the application follows.

SEQUENCE LISTING (15 sequences)

SEQ ID NO: 1 - protein, 847 aa, synthetic construct
MSSSSWLLLSLVAVTAAQSTIEEQAKTFLDKFNHEAEDLFYQSSLASWNYNTNITEENVQNMNNAGDKWSAFLKEQSTLAQMYPLQEIQNLTVKLQLQALQQNGSSVLSEDKSKRLNTILNTMSTIYSTGKVCNPDNPQECLLLEPGLNEIMANSLDYNERLWAWESWRSEVGKQLRPLYEEYVVLKNEMARANHYEDYGDYWRGDYEVNGVDGYDYSRGQLIEDVEHTFEEIKPLYEHLHAYVRAKLMNAYPSYISPIGCLPAHLLGDMWGRFWTNLYSLTVPFGQKPNIDVTDAMVDQAWDAQRIFKEAEKFFVSVGLPNMTQGFWENSMLTDPGNVQKAVCAPTAWDLGKGDFRILMCTKVTMDDFLTAHHEMGHIQYDMAYAAQPFLLRNGANEGFHEAVGEIMSLSAATPKHLKSIGLLSPDFQEDNETEINFLLKQALTIVGTLPFTYMLEKWRWMVFKGEIPKDQWMKKWWEMKREIVGVVEPVPHDETYCDPASLFAVSNDYSFIRYYTRTLYQFQFQEALCQAAKHEGPLHKCDISNSTEAGQKLFNMLRLGKSEPWTLALENVVGAKNMNVRPLLNYFEPLFTWLKDQNKNSFVGWSTDWSPYADEPKSCDKTHTCPPCPAPELLGGPSVFLFPPKPKDTLMISRTPEVTCVVVDVSHEDPEVKFNWYVDGVEVHNAKTKPREEQYNSTYRVVSVLTVLHQDWLNGKEYKCKVSNKALPAPIEKTISKAKGQPREPQVYTLPPSRDELTKNQVSLTCLVKGFYPSDIAVEWESNGQPENNYKTTPPVLDSDGSFFLYSKLTVDKSRWQQGNVFSCSVMHEALHNHYTQKSLSLSPGK

SEQ ID NO: 2 - DNA, 2547 bp, synthetic construct
  source 1..2547: mol_type = other DNA
atgagcagcagctcttggctgctgctgagtctggtggctgtgacagccgctcagagcaccattgaggaacaggccaagaccttcctggacaagttcaaccacgaggccgaggacctgttctaccagtctagcctggccagctggaactacaacaccaacatcaccgaagagaacgtgcagaacatgaacaacgccggcgacaagtggagcgccttcctgaaagagcagagcacactggcccagatgtaccctctgcaagagatccagaacctgaccgtgaagctccagctgcaggccctccagcagaatggaagctctgtgctgagcgaggacaagagcaagcggctgaacaccatcctgaataccatgtccaccatctacagcaccggcaaagtgtgcaaccccgacaatccccaagagtgcctgctgctggaacccggcctgaatgagatcatggccaacagcctggactacaacgagagactgtgggcctgggagtcttggagaagcgaagtgggaaagcagctgcggcccctgtacgaggaatacgtggtgctgaagaacgagatggccagagccaaccactacgaggactacggcgactattggagaggcgactacgaagtgaatggcgtggacggctacgactacagcagaggccagctgatcgaggacgtggaacacaccttcgaggaaatcaagcctctgtacgagcatctgcacgcctacgtgcgggccaagctgatgaatgcttaccccagctacatcagccccatcggctgtctgcctgctcatctgctgggagacatgtggggcagattctggaccaacctgtacagcctgacagtgcccttcggccagaaacctaacatcgacgtgaccgacgccatggtggatcaggcttgggatgcccagcggatcttcaaagaggccgagaagttcttcgtgtccgtgggcctgcctaatatgacccaaggcttctgggagaactccatgctgacagaccccggcaatgtgcagaaagccgtgtgtgctcctaccgcctgggatctcggaaagggcgacttcagaatcctgatgtgcaccaaagtgacgatggacgacttcctgacagcccaccacgagatgggccacatccagtacgatatggcctacgccgctcagcccttcctgctgagaaatggcgccaatgagggcttccacgaagccgtgggagagatcatgagcctgtctgccgccacacctaagcacctgaagtctatcggactgctgagccccgacttccaagaggacaacgagacagagatcaacttcctgctcaagcaggccctgaccatcgtgggcacactgcccttcacctacatgctggaaaagtggcggtggatggtctttaagggcgagatccccaaggaccagtggatgaagaaatggtgggagatgaagcgcgagatcgtgggcgttgtggaacctgtgcctcacgacgagacatactgcgatcctgccagcctgttcgccgtgtccaacgactactccttcatccggtactacacccggacactgtaccagttccagtttcaagaggctctgtgccaggccgccaagcacgaaggacctctgcacaagtgcgacatcagcaactctacagaggccggacagaaactgttcaacatgctgcggctgggcaagagcgagccttggacactggctctggaaaatgtcgtgggcgccaagaatatgaacgtgcggccactgctgaactacttcgagcccctgttcacctggctgaaggaccagaacaagaacagcttcgtcggctggtccaccgattggagcccttatgccgatgagcccaagtcctgcgacaagacccacacctgtcctccatgtcctgctccagaactgctcggcggaccttccgtgttcctgtttcctccaaagcctaaggacaccctgatgatcagcagaacccctgaagtgacctgcgtggtggtggatgtgtcccacgaggatcccgaagtgaagttcaattggtacgtcgacggcgtggaagtgcacaacgccaagaccaagcctagagaggaacagtacaacagcacctacagagtggtgtccgtgctgaccgtgctgcaccaggattggctgaacggcaaagagtacaagtgcaaggtgtccaacaaggccctgccagctcctatcgagaaaaccatcagcaaggccaagggccagcctagggaaccccaggtttacacactgcctccaagcagggacgagctgaccaagaatcaggtgtccctgacctgcctggtcaagggcttctacccttccgatatcgccgtggaatgggagagcaatggccagcctgagaacaactacaagacaacccctcctgtgctggacagcgacggctcattcttcctgtactccaaactgaccgtggacaagtccagatggcagcagggcaacgtgttcagctgcagcgtgctgcatgaagccctgcacagccactacacccagaagtccctgtctctgagccctggcaagtgatga

SEQ ID NO: 3 - protein, 847 aa, synthetic construct
MSSSSWLLLSLVAVTAAQSTIEEQAKFFLDWFNHEAEDLFYQMSLASWNYNTNITEENVQNMNNAGDKWSAFLKEQSTLASMYPLQEIQNLTVKLQLQALQQNGSSVLSEDKSKRLNTILNTMSTIYSTGKVCNPDNPQECLLLEPGLNEIMANSLDYNERLWAWESWRSEVGKQLRPLYEEYVVLKNEMARANHYEDYGDYWRGDYEVNGVDGYDYSRGQLIEDVEHTFEEIKPLYEHLHAYVRAKLMNAYPSYISPIGCLPAHLLGDMWGRFWTNLYSLTVPFGQKPNIDVTDAMVDQAWDAQRIFKEAEKFFVSVGLPNMTQGFWENSMLTDPGNVQKAVCAPTAWDLGKGDFRILMCTKVTMDDFLTAHHEMGHIQYDMAYAAQPFLLRNGANEGFHEAVGEIMSLSAATPKHLKSIGLLSPDFQEDNETEINFLLKQALTIVGTLPFTYMLEKWRWMVFKGEIPKDQWMKKWWEMKREIVGVVEPVPHDETYCDPASLFAVSNDYSFIRYYTRTLYQFQFQEALCQAAKHEGPLHKCDISNSTEAGQKLFNMLRLGKSEPWTLALENVVGAKNMNVRPLLNYFEPLFTWLKDQNKNSFVGWSTDWSPYADEPKSCDKTHTCPPCPAPELLGGPSVFLFPPKPKDTLMISRTPEVTCVVVDVSHEDPEVKFNWYVDGVEVHNAKTKPREEQYNSTYRVVSVLTVLHQDWLNGKEYKCKVSNKALPAPIEKTISKAKGQPREPQVYTLPPSRDELTKNQVSLTCLVKGFYPSDIAVEWESNGQPENNYKTTPPVLDSDGSFFLYSKLTVDKSRWQQGNVFSCSVMHEALHNHYTQKSLSLSPGK

SEQ ID NO: 4 - DNA, 2547 bp, synthetic construct
  source 1..2547: mol_type = other DNA
atgagcagcagctcttggctgctgctgagtctggtggctgtgacagccgctcagagcaccattgaggaacaggccaagttcttcctggactggttcaaccacgaggccgaggacctgttctaccagatgtctctggccagctggaactacaacaccaacatcaccgaagagaacgtgcagaacatgaacaacgccggcgacaagtggagcgccttcctgaaagagcagagcaccctggccagcatgtaccctctgcaggaaatccagaacctgaccgtgaagctccagctgcaagccctccagcagaatggcagctctgtgctgagcgaggacaagagcaagcggctgaacaccatcctgaataccatgtccaccatctacagcaccggcaaagtgtgcaaccccgacaatccccaagagtgcctgctgctggaacccggcctgaatgagatcatggccaacagcctggactacaacgagaggctgtgggcctgggagtcttggagatctgaagtgggcaagcagctgcggcccctgtacgaggaatatgtggtgctgaagaacgagatggccagagccaaccactacgaggactacggcgactattggagaggcgactacgaagtgaatggcgtggacggctacgactacagcagaggccagctgatcgaggacgtggaacacaccttcgaggaaatcaagcctctgtacgagcatctgcacgcctacgtgcgggccaagctgatgaatgcttaccccagctacatcagccccatcggctgtctgcctgctcatctgctgggagacatgtggggcagattctggaccaacctgtacagcctgacagtgcccttcggccagaaacctaacatcgacgtgaccgacgccatggtggatcaggcttgggatgcccagcggatcttcaaagaggccgaaaagttcttcgtgtccgtgggcctgcctaatatgacccaaggcttctgggagaactccatgctgacagaccccggcaatgtgcagaaagccgtgtgtgctcctaccgcctgggatctcggaaagggcgacttcagaatcctgatgtgcaccaaagtgacgatggacgacttcctgacagcccaccacgagatgggccacatccagtacgatatggcctacgccgctcagcccttcctgctgagaaatggcgccaatgagggcttccacgaagccgtgggagagatcatgagcctgtctgccgccacacctaagcacctgaagtctatcggactgctgagccccgacttccaagaggacaacgagacagagatcaacttcctgctcaagcaggccctgaccatcgtgggcacactgcccttcacctatatgctggaaaagtggcggtggatggtctttaagggcgagatccccaaggaccagtggatgaagaaatggtgggagatgaagcgcgagatcgtgggcgttgtggaacctgtgcctcacgacgagacatactgcgatcctgccagcctgttcgccgtgtccaacgactactccttcatccggtactacacccggacactgtaccagttccagtttcaagaggctctgtgccaggccgccaagcacgaaggacctctgcacaagtgcgacatcagcaactctacagaggccggacagaaactgttcaacatgctgcggctgggcaagagcgagccttggacactggccctggaaaatgttgtgggcgccaagaatatgaacgtgcggccactgctgaactacttcgagcccctgttcacctggctgaaggaccagaacaagaacagcttcgtcggctggtccaccgattggagcccttatgccgatgagcccaagtcctgcgacaagacccacacctgtcctccatgtcctgctccagaactgctcggcggaccttccgtgttcctgtttcctccaaagcctaaggacaccctgatgatcagcagaacccctgaagtgacctgcgtggtggtggatgtgtcccacgaggatcccgaagtgaagttcaattggtacgtcgacggcgtggaagtgcacaacgccaagaccaagcctagagaggaacagtacaacagcacctacagagtggtgtccgtgctgaccgtgctgcaccaggattggctgaacggcaaagagtacaagtgcaaggtgtccaacaaggccctgccagctcctatcgagaaaaccatcagcaaggccaagggccagcctagggaaccccaggtttacacactgcctccaagcagggacgagctgaccaagaatcaggtgtccctgacctgcctggtcaagggcttctacccttccgatatcgccgtggaatgggagagcaatggccagcctgagaacaactacaagacaacccctcctgtgctggacagcgacggctcattcttcctgtactccaaactgaccgtggacaagtccagatggcagcagggcaacgtgttcagctgctccgtgatgcacgaggccctgcacaatcactacacccagaagtccctgtctctgagccctggcaagtgatga

SEQ ID NO: 5 - protein, 887 aa, synthetic construct
MSSSSWLLLSLVAVTAAQSTIEEQAKTFLDKFNHEAEDLFYQSSLASWNYNTNITEENVQNMNNAGDKWSAFLKEQSTLAQMYPLQEIQNLTVKLQLQALQQNGSSVLSEDKSKRLNTILNTMSTIYSTGKVCNPDNPQECLLLEPGLNEIMANSLDYNERLWAWESWRSEVGKQLRPLYEEYVVLKNEMARANHYEDYGDYWRGDYEVNGVDGYDYSRGQLIEDVEHTFEEIKPLYEHLHAYVRAKLMNAYPSYISPIGCLPAHLLGDMWGRFWTNLYSLTVPFGQKPNIDVTDAMVDQAWDAQRIFKEAEKFFVSVGLPNMTQGFWENSMLTDPGNVQKAVCAPTAWDLGKGDFRILMCTKVTMDDFLTAHHEMGHIQYDMAYAAQPFLLRNGANEGFHEAVGEIMSLSAATPKHLKSIGLLSPDFQEDNETEINFLLKQALTIVGTLPFTYMLEKWRWMVFKGEIPKDQWMKKWWEMKREIVGVVEPVPHDETYCDPASLFAVSNDYSFIRYYTRTLYQFQFQEALCQAAKHEGPLHKCDISNSTEAGQKLFNMLRLGKSEPWTLALENVVGAKNMNVRPLLNYFEPLFTWLKDQNKNSFVGWSTDWSPYADGGGSGGGSGGGSGGGSGGGSGGGSGGGSGGGSGGGSGGGSEPKSCDKTHTCPPCPAPELLGGPSVFLFPPKPKDTLMISRTPEVTCVVVDVSHEDPEVKFNWYVDGVEVHNAKTKPREEQYNSTYRVVSVLTVLHQDWLNGKEYKCKVSNKALPAPIEKTISKAKGQPREPQVYTLPPSRDELTKNQVSLTCLVKGFYPSDIAVEWESNGQPENNYKTTPPVLDSDGSFFLYSKLTVDKSRWQQGNVFSCSVMHEALHNHYTQKSLSLSPGK

SEQ ID NO: 6 - DNA, 2667 bp, synthetic construct
  source 1..2667: mol_type = other DNA
atgagcagcagctcttggctgctgctgagtctggtggctgtgacagccgctcagagcaccattgaggaacaggccaagaccttcctggacaagttcaaccacgaggccgaggacctgttctaccagtctagcctggccagctggaactacaacaccaacatcaccgaagagaacgtgcagaacatgaacaacgccggcgacaagtggagcgccttcctgaaagagcagagcacactggcccagatgtaccctctgcaagagatccagaacctgaccgtgaagctccagctgcaggccctccagcagaatggaagctctgtgctgagcgaggacaagagcaagcggctgaacaccatcctgaataccatgtccaccatctacagcaccggcaaagtgtgcaaccccgacaatccccaagagtgcctgctgctggaacccggcctgaatgagatcatggccaacagcctggactacaacgagagactgtgggcctgggagtcttggagaagcgaagtgggaaagcagctgcggcccctgtacgaggaatacgtggtgctgaagaacgagatggccagagccaaccactacgaggactacggcgactattggagaggcgactacgaagtgaatggcgtggacggctacgactacagcagaggccagctgatcgaggacgtggaacacaccttcgaggaaatcaagcctctgtacgagcatctgcacgcctacgtgcgggccaagctgatgaatgcttaccccagctacatcagccccatcggctgtctgcctgctcatctgctgggagacatgtggggcagattctggaccaacctgtacagcctgacagtgcccttcggccagaaacctaacatcgacgtgaccgacgccatggtggatcaggcttgggatgcccagcggatcttcaaagaggccgagaagttcttcgtgtccgtgggcctgcctaatatgacccaaggcttctgggagaactccatgctgacagaccccggcaatgtgcagaaagccgtgtgtgctcctaccgcctgggatctcggaaagggcgacttcagaatcctgatgtgcaccaaagtgaccatggacgactttctgacagcccaccacgagatgggccacatccagtacgatatggcctacgccgctcagcccttcctgctgagaaatggcgccaatgagggcttccacgaggccgtgggagagatcatgtctctgtctgccgccacacctaagcacctgaagtctatcggactgctgagccccgacttccaagaggacaacgagacagagatcaacttcctgctcaagcaggccctgaccatcgtgggcacactgcccttcacctacatgctggaaaagtggcggtggatggtgttcaagggcgagatccccaaggaccagtggatgaagaaatggtgggagatgaagcgcgagatcgtgggcgttgtggaacccgtgcctcacgacgagacatactgtgatcctgccagcctgttcgccgtgtccaacgactacagcttcatccggtactacacccggacactgtaccagttccagtttcaagaggctctgtgccaggccgccaagcacgaaggacctctgcacaagtgcgacatcagcaactctacagaggccggccagaaactgttcaacatgctgagactgggcaagagcgagccctggacactggccctggaaaatgttgtgggcgccaagaacatgaacgtgcggcccctgctgaactacttcgagcctctgttcacctggctgaaggaccagaacaagaacagcttcgtcggctggtccaccgattggagcccttatgctgatggcggaggttctggcggaggaagcggtggcggatcaggtggtggaagcggcggtggtagtggtggtggatcaggcggcggtagcggaggcggctctggcggtggctccggcggaggctctgaacctaagagctgcgacaagacccacacctgtcctccatgtcctgctccagaactgctcggcggaccttccgtgttcctgtttcctccaaagcctaaggacaccctgatgatcagcagaacccctgaagtgacctgcgtggtggtcgatgtgtctcacgaggatcccgaagtgaagttcaattggtacgtcgacggcgtggaagtgcacaacgccaagaccaagcctagagaggaacagtacaacagcacctacagagtggtgtccgtgctgaccgtgctgcaccaggattggctgaacggcaaagagtacaagtgcaaggtgtccaacaaggccctgccagctcctatcgagaaaaccatcagcaaggccaagggccagcctagggaaccccaggtttacacactgcctccaagcagggacgagctgaccaagaatcaggtgtccctgacctgcctggtcaagggcttctacccttccgatatcgccgtggaatgggagagcaatggccagcctgagaacaactacaagacaacccctcctgtgctggacagcgacggctcattcttcctgtactccaaactgaccgtggacaagtccagatggcagcagggcaacgtgttcagctgcagcgtgctgcatgaagccctgcacagccactacacccagaagtccctgtctctgagccctggcaagtgatga

SEQ ID NO: 7 - protein, 887 aa, synthetic construct
MSSSSWLLLSLVAVTAAQSTIEEQAKFFLDWFNHEAEDLFYQMSLASWNYNTNITEENVQNMNNAGDKWSAFLKEQSTLASMYPLQEIQNLTVKLQLQALQQNGSSVLSEDKSKRLNTILNTMSTIYSTGKVCNPDNPQECLLLEPGLNEIMANSLDYNERLWAWESWRSEVGKQLRPLYEEYVVLKNEMARANHYEDYGDYWRGDYEVNGVDGYDYSRGQLIEDVEHTFEEIKPLYEHLHAYVRAKLMNAYPSYISPIGCLPAHLLGDMWGRFWTNLYSLTVPFGQKPNIDVTDAMVDQAWDAQRIFKEAEKFFVSVGLPNMTQGFWENSMLTDPGNVQKAVCAPTAWDLGKGDFRILMCTKVTMDDFLTAHHEMGHIQYDMAYAAQPFLLRNGANEGFHEAVGEIMSLSAATPKHLKSIGLLSPDFQEDNETEINFLLKQALTIVGTLPFTYMLEKWRWMVFKGEIPKDQWMKKWWEMKREIVGVVEPVPHDETYCDPASLFAVSNDYSFIRYYTRTLYQFQFQEALCQAAKHEGPLHKCDISNSTEAGQKLFNMLRLGKSEPWTLALENVVGAKNMNVRPLLNYFEPLFTWLKDQNKNSFVGWSTDWSPYADGGGSGGGSGGGSGGGSGGGSGGGSGGGSGGGSGGGSGGGSEPKSCDKTHTCPPCPAPELLGGPSVFLFPPKPKDTLMISRTPEVTCVVVDVSHEDPEVKFNWYVDGVEVHNAKTKPREEQYNSTYRVVSVLTVLHQDWLNGKEYKCKVSNKALPAPIEKTISKAKGQPREPQVYTLPPSRDELTKNQVSLTCLVKGFYPSDIAVEWESNGQPENNYKTTPPVLDSDGSFFLYSKLTVDKSRWQQGNVFSCSVMHEALHNHYTQKSLSLSPGK

SEQ ID NO: 8 - DNA, 2667 bp, synthetic construct
  source 1..2667: mol_type = other DNA
atgagcagcagctcttggctgctgctgagtctggtggctgtgacagccgctcagagcaccattgaggaacaggccaagttcttcctggactggttcaaccacgaggccgaggacctgttctaccagatgtctctggccagctggaactacaacaccaacatcaccgaagagaacgtgcagaacatgaacaacgccggcgacaagtggagcgccttcctgaaagagcagagcaccctggccagcatgtaccctctgcaggaaatccagaacctgaccgtgaagctccagctgcaagccctccagcagaatggcagctctgtgctgagcgaggacaagagcaagcggctgaacaccatcctgaataccatgtccaccatctacagcaccggcaaagtgtgcaaccccgacaatccccaagagtgcctgctgctggaacccggcctgaatgagatcatggccaacagcctggactacaacgagaggctgtgggcctgggagtcttggagatctgaagtgggcaagcagctgcggcccctgtacgaggaatatgtggtgctgaagaacgagatggccagagccaaccactacgaggactacggcgactattggagaggcgactacgaagtgaatggcgtggacggctacgactacagcagaggccagctgatcgaggacgtggaacacaccttcgaggaaatcaagcctctgtacgagcatctgcacgcctacgtgcgggccaagctgatgaatgcttaccccagctacatcagccccatcggctgtctgcctgctcatctgctgggagacatgtggggcagattctggaccaacctgtacagcctgacagtgcccttcggccagaaacctaacatcgacgtgaccgacgccatggtggatcaggcttgggatgcccagcggatcttcaaagaggccgaaaagttcttcgtgtccgtgggcctgcctaatatgacccaaggcttctgggagaactccatgctgacagaccccggcaatgtgcagaaagccgtgtgtgctcctaccgcctgggatctcggaaagggcgacttcagaatcctgatgtgcaccaaagtgaccatggacgactttctgacagcccaccacgagatgggccacatccagtacgatatggcctacgccgctcagcccttcctgctgagaaatggcgccaatgagggcttccacgaggccgtgggagagatcatgtctctgtctgccgccacacctaagcacctgaagtctatcggactgctgagccccgacttccaagaggacaacgagacagagatcaacttcctgctcaagcaggccctgaccatcgtgggcacactgcccttcacctacatgctggaaaagtggcggtggatggtgttcaagggcgagatccccaaggaccagtggatgaagaaatggtgggagatgaagcgcgagatcgtgggcgttgtggaacccgtgcctcacgacgagacatactgtgatcctgccagcctgttcgccgtgtccaacgactacagcttcatccggtactacacccggacactgtaccagttccagtttcaagaggctctgtgccaggccgccaagcacgaaggacctctgcacaagtgcgacatcagcaactctacagaggccggccagaaactgttcaacatgctgagactgggcaagagcgagccctggacactggccctggaaaatgttgtgggcgccaagaacatgaacgtgcggcccctgctgaactacttcgagcctctgttcacctggctgaaggaccagaacaagaacagcttcgtcggctggtccaccgattggagcccttatgctgatggcggaggttctggcggaggaagcggtggcggatcaggtggtggaagcggcggtggtagtggtggtggatcaggcggcggtagcggaggcggctctggcggtggctccggcggaggctctgaacctaagagctgcgacaagacccacacctgtcctccatgtcctgctccagaactgctcggcggaccttccgtgttcctgtttcctccaaagcctaaggacaccctgatgatcagcagaacccctgaagtgacctgcgtggtggtcgatgtgtctcacgaggatcccgaagtgaagttcaattggtacgtcgacggcgtggaagtgcacaacgccaagaccaagcctagagaggaacagtacaacagcacctacagagtggtgtccgtgctgaccgtgctgcaccaggattggctgaacggcaaagagtacaagtgcaaggtgtccaacaaggccctgccagctcctatcgagaaaaccatcagcaaggccaagggccagcctagggaaccccaggtttacacactgcctccaagcagggacgagctgaccaagaatcaggtgtccctgacctgcctggtcaagggcttctacccttccgatatcgccgtggaatgggagagcaatggccagcctgagaacaactacaagacaacccctcctgtgctggacagcgacggctcattcttcctgtactccaaactgaccgtggacaagtccagatggcagcagggcaacgtgttcagctgctccgtgatgcacgaggccctgcacaatcactacacccagaagtccctgtctctgagccctggcaagtgatga

SEQ ID NO: 9 - protein, 1525 aa, synthetic construct
MSSSSWLLLSLVAVTAAQSTIEEQAKTFLDKFNHEAEDLFYQSSLASWNYNTNITEENVQNMNNAGDKWSAFLKEQSTLAQMYPLQEIQNLTVKLQLQALQQNGSSVLSEDKSKRLNTILNTMSTIYSTGKVCNPDNPQECLLLEPGLNEIMANSLDYNERLWAWESWRSEVGKQLRPLYEEYVVLKNEMARANHYEDYGDYWRGDYEVNGVDGYDYSRGQLIEDVEHTFEEIKPLYEHLHAYVRAKLMNAYPSYISPIGCLPAHLLGDMWGRFWTNLYSLTVPFGQKPNIDVTDAMVDQAWDAQRIFKEAEKFFVSVGLPNMTQGFWENSMLTDPGNVQKAVCAPTAWDLGKGDFRILMCTKVTMDDFLTAHHEMGHIQYDMAYAAQPFLLRNGANEGFHEAVGEIMSLSAATPKHLKSIGLLSPDFQEDNETEINFLLKQALTIVGTLPFTYMLEKWRWMVFKGEIPKDQWMKKWWEMKREIVGVVEPVPHDETYCDPASLFAVSNDYSFIRYYTRTLYQFQFQEALCQAAKHEGPLHKCDISNSTEAGQKLFNMLRLGKSEPWTLALENVVGAKNMNVRPLLNYFEPLFTWLKDQNKNSFVGWSTDWSPYADGGGSGGGSGGGSGGGSGGGSGGGSGGGSGGGSGGGSGGGSEPKSCDKTHTCPPCPAPELLGGPSVFLFPPKPKDTLMISRTPEVTCVVVDVSHEDPEVKFNWYVDGVEVHNAKTKPREEQYNSTYRVVSVLTVLHQDWLNGKEYKCKVSNKALPAPIEKTISKAKGQPREPQVYTLPPSRDELTKNQVSLTCLVKGFYPSDIAVEWESNGQPENNYKTTPPVLDSDGSFFLYSKLTVDKSRWQQGNVFSCSVMHEALHNHYTQKSLSLSPGKGGGSGGGSGGGSGGGSGGGSGGGSGGGSGGGSGGGSGGGSQSTIEEQAKTFLDKFNHEAEDLFYQSSLASWNYNTNITEENVQNMNNAGDKWSAFLKEQSTLAQMYPLQEIQNLTVKLQLQALQQNGSSVLSEDKSKRLNTILNTMSTIYSTGKVCNPDNPQECLLLEPGLNEIMANSLDYNERLWAWESWRSEVGKQLRPLYEEYVVLKNEMARANHYEDYGDYWRGDYEVNGVDGYDYSRGQLIEDVEHTFEEIKPLYEHLHAYVRAKLMNAYPSYISPIGCLPAHLLGDMWGRFWTNLYSLTVPFGQKPNIDVTDAMVDQAWDAQRIFKEAEKFFVSVGLPNMTQGFWENSMLTDPGNVQKAVCAPTAWDLGKGDFRILMCTKVTMDDFLTAHHEMGHIQYDMAYAAQPFLLRNGANEGFHEAVGEIMSLSAATPKHLKSIGLLSPDFQEDNETEINFLLKQALTIVGTLPFTYMLEKWRWMVFKGEIPKDQWMKKWWEMKREIVGVVEPVPHDETYCDPASLFAVSNDYSFIRYYTRTLYQFQFQEALCQAAKHEGPLHKCDISNSTEAGQKLFNMLRLGKSEPWTLALENVVGAKNMNVRPLLNYFEPLFTWLKDQNKNSFVGWSTDWSPYAD

SEQ ID NO: 10 - DNA, 4581 bp, synthetic construct
  source 1..4581: mol_type = other DNA
atgagcagcagctcttggctgctgctgagtctggtggctgtgacagccgctcagagcaccattgaggaacaggccaagttcttcctggactggttcaaccacgaggccgaggacctgttctaccagatgtctctggccagctggaactacaacaccaacatcaccgaagagaacgtgcagaacatgaacaacgccggcgacaagtggagcgccttcctgaaagagcagagcaccctggccagcatgtaccctctgcaggaaatccagaacctgaccgtgaagctccagctgcaagccctccagcagaatggcagctctgtgctgagcgaggacaagagcaagcggctgaacaccatcctgaataccatgtccaccatctacagcaccggcaaagtgtgcaaccccgacaatccccaagagtgcctgctgctggaacccggcctgaatgagatcatggccaacagcctggactacaacgagaggctgtgggcctgggagtcttggagatctgaagtgggcaagcagctgcggcccctgtacgaggaatatgtggtgctgaagaacgagatggccagagccaaccactacgaggactacggcgactattggagaggcgactacgaagtgaatggcgtggacggctacgactacagcagaggccagctgatcgaggacgtggaacacaccttcgaggaaatcaagcctctgtacgagcatctgcacgcctacgtgcgggccaagctgatgaatgcttaccccagctacatcagccccatcggctgtctgcctgctcatctgctgggagacatgtggggcagattctggaccaacctgtacagcctgacagtgcccttcggccagaaacctaacatcgacgtgaccgacgccatggtggatcaggcttgggatgcccagcggatcttcaaagaggccgaaaagttcttcgtgtccgtgggcctgcctaatatgacccaaggcttctgggagaactccatgctgacagaccccggcaatgtgcagaaagccgtgtgtgctcctaccgcctgggatctcggaaagggcgacttcagaatcctgatgtgcaccaaagtgaccatggacgactttctgacagcccaccacgagatgggccacatccagtacgatatggcctacgccgctcagcccttcctgctgagaaatggcgccaatgagggcttccacgaggccgtgggagagatcatgtctctgtctgccgccacacctaagcacctgaagtctatcggactgctgagccccgacttccaagaggacaacgagacagagatcaacttcctgctcaagcaggccctgaccatcgtgggcacactgcccttcacctacatgctggaaaagtggcggtggatggtgttcaagggcgagatccccaaggaccagtggatgaagaaatggtgggagatgaagcgcgagatcgtgggcgttgtggaacccgtgcctcacgacgagacatactgtgatcctgccagcctgttcgccgtgtccaacgactacagcttcatccggtactacacccggacactgtaccagttccagtttcaagaggctctgtgccaggccgccaagcacgaaggacctctgcacaagtgcgacatcagcaactctacagaggccggccagaaactgttcaacatgctgagactgggcaagagcgagccctggacactggccctggaaaatgttgtgggcgccaagaacatgaacgtgcggcccctgctgaactacttcgagcctctgttcacctggctgaaggaccagaacaagaacagcttcgtcggctggtccaccgattggagcccttatgctgatggcggaggttctggcggaggaagcggtggcggatcaggtggtggaagcggcggtggtagtggtggtggatcaggcggcggtagcggaggcggctctggcggtggctccggcggaggctctgaacctaagagctgcgacaagacccacacctgtcctccatgtcctgctccagaactgctcggcggaccttccgtgttcctgtttcctccaaagcctaaggacaccctgatgatcagcagaacccctgaagtgacctgcgtggtggtcgatgtgtctcacgaggatcccgaagtgaagttcaattggtacgtggacggcgtggaagtgcacaacgccaagaccaagcctagagaggaacagtacaacagcacctacagagtggtgtccgtgctgaccgtgctgcaccaggattggctgaacggcaaagagtacaagtgcaaggtgtccaacaaggccctgcctgctcctatcgagaaaaccatcagcaaggccaagggccagcctagggaaccccaggtttacacactgcctccaagcagggacgagctgaccaagaatcaggtgtccctgacctgcctggtcaagggcttctacccttccgatatcgccgtggaatgggagagcaacggccagcctgagaacaactacaagacaacccctcctgtgctggacagcgacggctcattcttcctgtacagcaagctgacagtggacaagagcagatggcagcagggcaacgtgttcagctgcagcgtgatgcacgaggccctgcacaaccactacacccagaagtccctgagcctgtctcctggcaaaggcggaggaagtggtggcggatctggcggtggttctggcggcggaagcggcggaggctctggcggaggtagcggaggtggaagcggtggtggcagcggcggtggatcaggcggtggctctcaaagcacaatcgaggaacaggccaagttcttcctggactggttcaaccacgaggccgaggacctgttctaccagatgtctctggccagctggaactacaacaccaacatcaccgaagagaacgtgcagaacatgaacaacgccggcgacaagtggagcgccttcctgaaagagcagagcaccctggccagcatgtaccctctgcaagagatccagaacctgaccgtgaagctgcaactgcaggctctgcagcagaatggctctagcgtgctgagcgaggacaagtccaagcggctgaacaccatcctgaataccatgagcaccatctacagcaccggcaaagtgtgcaaccccgacaatccccaagagtgcctgctgctggaacccggcctgaatgagatcatggccaacagcctggactacaacgagagactgtgggcctgggagtcttggagaagcgaagtgggaaagcagctgcggcccctgtacgaggaatacgtggtgctgaagaacgagatggccagagccaatcactacgaggactacggcgactactggcggggagactacgaagtgaatggcgtggacggatacgactacagcagaggccagctgatcgaggacgtggaacacaccttcgaggaaatcaagcctctgtacgagcatctgcacgcctacgtgcgggccaagctgatgaatgcttaccccagctacatcagccccatcggctgtctgccagctcatctgctgggagacatgtggggcagattctggaccaacctgtactccctgacagtgcccttcggccagaaacctaacatcgacgtgaccgacgccatggtggaccaggcttgggatgcccagcggatcttcaaagaggccgagaagttcttcgtgtccgtgggcctgcctaatatgacccaaggcttctgggagaactccatgctgacagaccccggcaatgtgcagaaagccgtgtgtgctcctaccgcctgggatctcggaaagggcgacttcagaatcctgatgtgcaccaaagtgacgatggacgacttcctgacagcccaccacgagatgggccacatccagtacgatatggcctacgccgctcagcccttcctgctgagaaatggcgccaatgagggcttccacgaagccgtgggagagatcatgtctctgtctgccgccacacctaagcacctgaagtctatcggactgctgagccccgacttccaagaggacaacgagacagagatcaacttcctgctcaagcaggccctgaccatcgtgggcaccctgcctttcacctatatgctggaaaagtggcgctggatggtctttaagggcgagatccccaaggaccagtggatgaagaaatggtgggagatgaagcgcgagatcgtgggcgttgtggaacctgtgcctcacgacgagacatactgcgatcctgccagcctgttcgccgtgtccaacgactactccttcatccggtactacacccggacactgtaccagttccagtttcaagaggctctgtgccaggccgccaagcacgaaggacctctgcacaagtgcgacatcagcaactctacagaggccggacagaaactgttcaacatgctgcggctgggcaagagcgagccttggacactggccctggaaaatgttgtgggcgccaagaatatgaacgtgcggccactgctgaactacttcgagcccctgttcacctggctgaaggaccagaacaagaacagcttcgtcggctggtctaccgattggagcccctacgccgattgatga

SEQ ID NO: 11 - protein, 1525 aa, synthetic construct
MSSSSWLLLSLVAVTAAQSTIEEQAKFFLDWFNHEAEDLFYQMSLASWNYNTNITEENVQNMNNAGDKWSAFLKEQSTLASMYPLQEIQNLTVKLQLQALQQNGSSVLSEDKSKRLNTILNTMSTIYSTGKVCNPDNPQECLLLEPGLNEIMANSLDYNERLWAWESWRSEVGKQLRPLYEEYVVLKNEMARANHYEDYGDYWRGDYEVNGVDGYDYSRGQLIEDVEHTFEEIKPLYEHLHAYVRAKLMNAYPSYISPIGCLPAHLLGDMWGRFWTNLYSLTVPFGQKPNIDVTDAMVDQAWDAQRIFKEAEKFFVSVGLPNMTQGFWENSMLTDPGNVQKAVCAPTAWDLGKGDFRILMCTKVTMDDFLTAHHEMGHIQYDMAYAAQPFLLRNGANEGFHEAVGEIMSLSAATPKHLKSIGLLSPDFQEDNETEINFLLKQALTIVGTLPFTYMLEKWRWMVFKGEIPKDQWMKKWWEMKREIVGVVEPVPHDETYCDPASLFAVSNDYSFIRYYTRTLYQFQFQEALCQAAKHEGPLHKCDISNSTEAGQKLFNMLRLGKSEPWTLALENVVGAKNMNVRPLLNYFEPLFTWLKDQNKNSFVGWSTDWSPYADGGGSGGGSGGGSGGGSGGGSGGGSGGGSGGGSGGGSGGGSEPKSCDKTHTCPPCPAPELLGGPSVFLFPPKPKDTLMISRTPEVTCVVVDVSHEDPEVKFNWYVDGVEVHNAKTKPREEQYNSTYRVVSVLTVLHQDWLNGKEYKCKVSNKALPAPIEKTISKAKGQPREPQVYTLPPSRDELTKNQVSLTCLVKGFYPSDIAVEWESNGQPENNYKTTPPVLDSDGSFFLYSKLTVDKSRWQQGNVFSCSVMHEALHNHYTQKSLSLSPGKGGGSGGGSGGGSGGGSGGGSGGGSGGGSGGGSGGGSGGGSQSTIEEQAKFFLDWFNHEAEDLFYQMSLASWNYNTNITEENVQNMNNAGDKWSAFLKEQSTLASMYPLQEIQNLTVKLQLQALQQNGSSVLSEDKSKRLNTILNTMSTIYSTGKVCNPDNPQECLLLEPGLNEIMANSLDYNERLWAWESWRSEVGKQLRPLYEEYVVLKNEMARANHYEDYGDYWRGDYEVNGVDGYDYSRGQLIEDVEHTFEEIKPLYEHLHAYVRAKLMNAYPSYISPIGCLPAHLLGDMWGRFWTNLYSLTVPFGQKPNIDVTDAMVDQAWDAQRIFKEAEKFFVSVGLPNMTQGFWENSMLTDPGNVQKAVCAPTAWDLGKGDFRILMCTKVTMDDFLTAHHEMGHIQYDMAYAAQPFLLRNGANEGFHEAVGEIMSLSAATPKHLKSIGLLSPDFQEDNETEINFLLKQALTIVGTLPFTYMLEKWRWMVFKGEIPKDQWMKKWWEMKREIVGVVEPVPHDETYCDPASLFAVSNDYSFIRYYTRTLYQFQFQEALCQAAKHEGPLHKCDISNSTEAGQKLFNMLRLGKSEPWTLALENVVGAKNMNVRPLLNYFEPLFTWLKDQNKNSFVGWSTDWSPYAD

SEQ ID NO: 12 - DNA, 4581 bp, synthetic construct; identical to SEQ ID NO: 10
  source 1..4581: mol_type = other DNA

SEQ ID NO: 13 - protein, 232 aa, Homo sapiens
EPKSCDKTHTCPPCPAPELLGGPSVFLFPPKPKDTLMISRTPEVTCVVVDVSHEDPEVKFNWYVDGVEVHNAKTKPREEQYNSTYRVVSVLTVLHQDWLNGKEYKCKVSNKALPAPIEKTISKAKGQPREPQVYTLPPSRDELTKNQVSLTCLVKGFYPSDIAVEWESNGQPENNYKTTPPVLDSDGSFFLYSKLTVDKSRWQQGNVFSCSVMHEALHNHYTQKSLSLSPGK

SEQ ID NO: 14 - protein, 17 aa, Homo sapiens
MSSSSWLLLSLVAVTAA

SEQ ID NO: 15 - protein, 40 aa, synthetic construct
GGGSGGGSGGGSGGGSGGGSGGGSGGGSGGGSGGGSGGGS